European Patent Specification EP 3 206 479 B1, published November 5, 2025. Title: Yield QTLs in cucumber plants. Applicant: Nunhems B.V. The sequence listing filed with the application follows.

SEQUENCE LISTING (30 sequences)

SEQ ID NO: 1 - DNA, 150 bp, Cucumis sativus
aaatttattaaagtctttttttctctctcgatcatatattatttatatatttgttatcttttaaccctttgaacgatatagttcttaattaaaagtataggagttgcaacaaaagatggaacagccataccatatccaaaaccaatccac

SEQ ID NO: 2 - DNA, 150 bp, Cucumis sativus
taaaaggtttaaatgtgatcataaagaattccatctatctatatttcatttattaatgttgtcaacagtaataagaagcatttaactctatgtaaaaagatgaaacaaacaaaaagtaactcataacttcaatagatttcttaccatctm

SEQ ID NO: 3 - DNA, 150 bp, Cucumis sativus
caaaaaaaaacaaaaatcaaaaaaaggaaattacataaaacctaaagccctaaaccctaattcgctaaaaaagagacctaattttacggaaaagaaaagaactaacctagagatgacgtggcatyagattttctctgggtcccattttaa

SEQ ID NO: 4 - DNA, 150 bp, Cucumis sativus
tattgtttttgtggacgtatgattatcttaaaaattacttctaatatatatttggtgaagcaagtttttctaaggttaaaataaacaatacctccaaacaacttagaaaaatgacttttattgatgtaatsaaaaaaataaaatgatctc

SEQ ID NO: 5 - DNA, 150 bp, Cucumis sativus
tcatasaatgatgataactttgtgagcaatgtaacacaaagttaggtttaaacttactttttttcatctaaattctgtcatttggtcatatggatacgtttgtttaaaaacaataataataaagtagrttagtgttaakgctatatagat

SEQ ID NO: 6 - DNA, 150 bp, Cucumis sativus
kcaaatgttttctcttctaattttttttaacataataaaagatagagtacaaatagaaatagtaaatcgaaaaataaaaactaaatattacgaattttgataaaactgaaggaacaacgaaatagaaaaagcaaggatgttgctgcaaat

SEQ ID NO: 7 - DNA, 150 bp, Cucumis sativus
catgtcaatctcaaagtctattcacaaaaaatacaccatttgagggaagagggataattacaaggaaaagaaaagcagtgactaagtgaaaacaaatacaagatttcattttccacttatgacttcaatttcaaagatctttcgrtctat

SEQ ID NO: 8 - DNA, 150 bp, Cucumis sativus
rcatcaacmaaaaaaaammaaaaaggatccatcttgttcaacacgattgccacttttccctttggtccatttggttggagagaaacaatcaaatattcagcaacaaagcctgaacatagactgaattatgggaagacattaaatctctca

SEQ ID NO: 9 - DNA, 150 bp, Cucumis sativus
tggtgcttccttttcctcactttttttttaaattatgaaatctcttaacagagtattcaaggaaaagaagtgtgctataaaataaaactctctaagactaaagatatctatttgataactacttttttctttttgtcatagacatagcta

SEQ ID NO: 10 - DNA, 150 bp, Cucumis sativus
ctgtaaaaatatatacctagttcctagattccaaccagacaagttagcagcagtagttaaagcttccctccaaagttgggtctttgtttggaacttaggctgatgtttggccagtgcttctccgaagctaccagtttgttttcgtatatc

SEQ ID NO: 11 - DNA, 150 bp, Cucumis sativus
tcgggataaktttgattttgaaaatccatttgttagaaattagaaagggtgcatctcaatttacacaaagcttaaacattctagttgggatgttctttttgtcaaccggaaaggagaaaaacatctaacaaaaatcgaaygattacattc

SEQ ID NO: 12 - DNA, 150 bp, Cucumis sativus
aatgcagtatgaaccagmgggagatgagctttcctgataatgatcttttgttttgattccaatggaccaaaaaaacatatggagaatgaaaactaaacaaaccaaataagaaggcatctagactagtgtttgccatgtactcatagacaa

SEQ ID NO: 13 - DNA, 150 bp, Cucumis sativus
aacataattataccttttaatcgctaccacctgttaccaacaattataagcttgatgtagggttggaataatgtaatcaaattccaaacataatagtacataaaaacaaaactattttatttatttgtttgttattyargtcaagatctt

SEQ ID NO: 14 - DNA, 150 bp, Cucumis sativus
atcwtgcactaaagcaaattaagactgtttttgcaaagttaaacaagcttgagaaacttcttgtagagtccctgggtaaagatttgagctgtgagttacggaattaagccagacagacaacccattgtcaacaccattttggtttaatct

SEQ ID NO: 15 - DNA, 150 bp, Cucumis sativus
tcttctctaaccaatgttagaswttgtttgtgtctaacatatgtatcatgtacacagcggctggcttgcgaaactggtctcctgaaaacaaagcagtcattgtaagtgaagttgagaagatagtttggccagccattgcagcaggcragg

SEQ ID NO: 16 - DNA, 150 bp, Cucumis sativus
aattaaacccataatttgataaagaaataaaattaaaagaagaaagagtgtgacgtggctttcccaaatcgaataatgggattccatctggaagcttccacagtgttctggatctctgttgttcttccagactcatccttctgaacccct

SEQ ID NO: 17 - DNA, 150 bp, Cucumis sativus
aatggaattatggttggayttttgttaataggtatgaaaacaaatttttatgtttccattaaaagggacgtccttctataatatatgcaaattaattaagggtattaagggtgagaaaaaattatatattaattgttggacatttgtatt

SEQ ID NO: 18 - DNA, 150 bp, Cucumis sativus
ataatagaagaggagggcatgagtggaagaaacaagttcatctgctgaagaagttttgatattgagttcataatcctgaagagattgcagattcatggtgtaaaatgctaacgagatttaagtcttattaggagattgtaaaagaaaaac

SEQ ID NO: 19 - DNA, 150 bp, Cucumis sativus
rtatgtataggattgcaggatgaytctttataggagtaatagtgggaggatcaacactaattttattgtttcacaacctctgcttttagaaggaaagcaattcatagatttaaataatctcccagtcggaaaattcatcattttgaatgg

SEQ ID NO: 20 - DNA, 150 bp, Cucumis sativus
aggtgaacttgtgacatagataaaaagaattattattttagggtttagaaagacacaactttactgctactataagtgtgagttccataaatgagagacaacattagaggacaccaacccaatttaaacctaaattaaaagggttagagc

SEQ ID NO: 21 - DNA, 150 bp, Cucumis sativus
ttcctcaacgatttgtagcctttgtgacggttgggagtgctgatacgggccaacttggaaaagatcttgagaaggcggcggtggcaggtgtagagagagcggttaatggtggcaacgacagcggagggggcattcttgattggagacttg

SEQ ID NO: 22 - DNA, 150 bp, Cucumis sativus
tttggcaaaactcagagaatcaagaaggatttgggcagctttttgtggtatcggaggagcagaagcttgattggccagacatgttctacataaccactctccctcttaatctaaggaagcctcatctttttcaaaggcttccaccaaaac

SEQ ID NO: 23 - DNA, 150 bp, Cucumis sativus
gaaaatakaattttcttcccaaagactcaaaatccacccatctccagccgtcatctctcacgaatttcgcacggaccctacaaaatacaattcttctccaacattataccgccactctctttttttatttctttattatttcaatatata

SEQ ID NO: 24 - DNA, 150 bp, Cucumis sativus
tgtaaaatttaatggcaaaaaacttatgaaacaaaacaagttattataatatttaatgaagatttttcttctttcgctttattataatatttggagatgttgaagacaaaatgcataaaattctaaatattggatggaaacgttggagca

SEQ ID NO: 25 - DNA, 150 bp, Cucumis sativus
aatgagagctatcataattattgcaataatattgttctttttatttggggctcttttaattttttttatgtattggtatttaagtaaaatcatttgagttaaatcactaacaaagaattgagaaattcaataatgaccaaagggaactga

SEQ ID NO: 26 - DNA, 150 bp, Cucumis sativus
cctctgtttcagcttccacaacttgtatgatcttgcacccttcaagctcttcgataccaggtgtgtgttttttccactataacctaaaccctcgcaatgtttcaagaaagggtatgtgtgtttttgtgattttattcagattgaactctc

SEQ ID NO: 27 - DNA, 150 bp, Cucumis sativus
gggattcatcatyatgtamgaagagtatcaacttgtagggatatttctttataacccagatcaatttcagttttaatagacgtgatcacacgtgagtatagcatgctctatttatgcataatgctaagcgagtggttttatctmygagga

SEQ ID NO: 28 - DNA, 150 bp, Cucumis sativus
acacaatttatctcttcttcaycactgggggacccggcaacacttctctttcttgtcgtcttcacgttctttaactaatttcacttctgccctgcttcaatagtaagtgttttgtctgtttttctgctgttttcattttttccttttttg

SEQ ID NO: 29 - DNA, 150 bp, Cucumis sativus
cataaattataagcatccaattacataaaataaagtccctaccaactttgttatgtggtcaaaacagtcatcttctatgtatatataactcattaatatatataagtttatattcctaaattggatttgtgtggatattataaaagttya

SEQ ID NO: 30 - DNA, 150 bp, Cucumis sativus
gatttgattttcttggtgcttgttgatctgttctgctaattaagcatatttttatgaaatttataccgtctgaatttaaattttaatgtggatgagttactaatattattggaagcttgcagatgttgtgagggatgatcctacgaacaa